European Patent Specification EP 3 421 486 B1, published September 27, 2023. Title: NOVEL VISTA-IG CONSTRUCTS AND THE USE OF VISTA-IG FOR THE TREATMENT OF AUTOIMMUNE, ALLERGIC AND INFLAMMATORY DISORDERS. Applicant: THE TRUSTEES OF DARTMOUTH COLLEGE KING'S COLLEGE LONDON. Application PCT/US13/047009. The sequence listing filed with the application follows.

SEQUENCE LISTING (75 sequences)

SEQ ID NO: 1 - DNA, 4795 bp, Mus musculus
gagcattcactctagcgagcgagcggcgtgtacagccggctccctgggctcctggagtcccgcttgctccaagcgcactccagcagtctctttctgctcttgcccggctcgacggcgacatgggtgtccccgcggtcccagaggccagcagcccgcgctggggaaccctgctccttgctattttcctggctgcatccagaggtctggtagcagccttcaaggtcaccactccatattctctctatgtgtgtcccgagggacagaatgccaccctcacctgcaggattctgggccccgtgtccaaagggcacgatgtgaccatctacaagacgtggtacctcagctcacgaggcgaggtccagatgtgcaaagaacaccggcccatacgcaacttcacattgcagcaccttcagcaccacggaagccacctgaaagccaacgccagccatgaccagccccagaagcatgggctagagctagcttctgaccaccacggtaacttctctatcaccctgcgcaatgtgaccccaagggacagcggcctctactgctgtctagtgatagaattaaaaaaccaccacccagaacaacggttctacgggtccatggagctacaggtacaggcaggcaaaggctcggggtccacatgcatggcgtctaatgagcaggacagtgacagcatcacggctgcggccctggccaccggcgcctgcatcgtgggaatcctctgcctcccccttatcctgctgctggtctataagcagagacaggtggcctctcaccgccgtgcccaggagttggtgaggatggacagcagcaacacccaaggaatcgaaaacccaggcttcgagaccactccacccttccaggggatgcctgaggccaagaccaggccgccactgtcctatgtggcccagcggcaaccttcggagtcaggacggtacctgctctctgaccccagcacacctctgtcgcctccaggccctggggacgtctttttcccatccctagatccagtccctgactcccctaactctgaagccatctaaaccagctggggaaccatgaaccatggtacctgggtcagggatatgtgcacttgatctatggctggcccttggacagtcttttaggcactgactccagcttccttgctcctgctctgagcctagactctgcttttacaagatgcacagaccctcccctatctctttcagacgctacttggggggcagggagaagatgttggattgctcatggctgttctcaagatcttgggatgctgagttctccctagagacttgacttcgacagccacagatgtcagatgacctgcatcctatgaacgtccggcttggcaagagcctttcttcatggaaaccagtagcccggaggggatgaggtaggcaccttgccaccctcccgggagagagacacaagatgtgagagactcctgctcactgtgggggtgtggctggcctgcttgtttgcctgaggatgctcctctgttggactgactctatccccctggattctggagcttggctggcctatgtcccaccagaggagcatctcagcagccttccaccagcaacctgagggcctgccagcttcgtggctctgggctctcattacctgtatggccgtccacagagctcagtggccagaggctttgaaacaggaagtacatgtcaggttcaggaaccactgtgagctcattagtgtcttgagcaatgtgaggcctggaccagtggacacggagggagggtggcgagaggatgatggggatgatgaggggaacacgctcccttcctgtccttgtcatccaccactaccactattcagtgtggagcagtggcaaaggtgaccgacctccacaatgtcctagtgatgctggaccatttctaagtgtgaaagagatgctattaaaaacagtatgtggcaatggctgccaacagctgagtggactggaggcactggctttaaggccctggaggtgcagggcccggtatggggatagggatgggagtttcagtgagggcctagggatcactccgcttctgaccactcttcttctgagcctcacctcagggtgaccttcaggcacacagaagagcttgcccctggtccgatactactcttggctctcatctccagggtttggcatgacctgggcacacagggggagtcttcagaaaggattttaaagcatgaaaagaaagggtagttcttgtgaggtagggatgggcagctgatgtttgagagtgaggagggatacggctgggcagatcactctccagtctctagagggaaagtagctctaagtctgggagagcagcagcccagtggtaccatatgtcttcttgcagcttccactggctgggctgaactgggcatgggtaggaaagctcctgttctgggcctgcagccagggagaaccccattcattccctgaggacagatgggtggggagagaagagagagtttcaggccgggaagcagcaataagctatctgctggggacccagacaagttgtctgatgaggtccaagatgtgggatgccagttatacctggggcttggggatccttagaggctttgtatcatcatcataggagtgtcggggtggccagggcatcaaagccatgacccctgttttatcctcagggtccactcttctgcaccatccattgctctagatctatgcagttactatagacagaatgtgttgttctgtttggctttggggataatggcctggcgaactgccagctgttcagtggcagggctgtgaggccagtcaaagactagaacccacagaccagctgaacgatgagtatagcctgtcccctgggggagcctgacctgtctccagccctaagcttcagacctcaccactcagatgacttctaagaatttgcctgtggggacccctgcatggctgcagctccgtggaaaggagaggaggcccccagcagaagaaccactcgcttcctgcccagcttcctcctgtagggctctaagtctcttcttcttgggaccctgcaagcaaaggcatgtcagcttggtggtttcctgttttgggtgaagttttgtgtggtccgggttctgtctacatccatgaacttggggtgctaccaccttgctgctgctgtagagacagctgcaggatcttagggtggaaaatggaggtgccctgaggtgctagcccttggggcaaaagatggggtggcaatgagacacagtggggaactgagttccccaagaggagggaggagccctgtagcctcaagggccatattgggttcctggtaccagcaaaagcctagagagcgaagtctgtattttgaggaggtaattgatccttacggaatccatcagaaatttggagcgggtgctttatctatctctggagggtctctacctatctccgatgaagctctccctgggcctgggatgggagaaaccaggaggaaaggtgtctgataaagcaggggcttcttgacaagccaaagggccactggtagctgttgtggaccgagctgaccctgctgaagtattgtagtgtgccttggaccaacttctcaaaagagcaaccccggggctaccctacttctgccaggaagaggcggagaaggggctgagaggcctggaaggggctagctccttctttgagaactgctccccggaggacttggaggaggcggctaggctacgggctgctgagggccctttgtctttcctaacctgggcactgttaggatgctccctcctggaaaaggctttcctgggtgtgagctagagcagtgtccatgccagcgctgaacctgccatggtgggagctgaactaaaaatttctcagggaactaaaataggcaaaagaggaactgggggaggagggtgccaggcaggatggggggaagggagggcagtgcaaaagtctcttgaaacacagacagcccagctgagtgccagtcccagatcacagagaatacggctcatctggctcatgttctgcatgcttgctgctttaccctggcactttccttctccaccatgagtgcgagtcctgggagtcctgggagggtgaggattaatgccagcctggggagcagatagctgacagagtccttgggtaactggcttgaaccaggacctcaggattccactctggggatctagctttgtctgggccagtgaagatctctataatggcattattgccaggggataaacatttcactgggttctgatctgttgggtgtggcttcctggaaaatatggtgagaggaattctgctaaggatacagttgataagaaagttctgagattgattagtaatgcctgccttggactcaggaagggaagtggcagtatgaatgccatgtcttaatcattttggttaaaatatgcttcccaaaagatttccacgtgtgttcttgtttatttgacatctgtctccatatcagtcttgaaagcctttctgtgtgtatatatatgatgtttgcgtgtatatatgtttttgtgtgtgcatatggaagtcagaaatcactgggtgtcttcctccattcctttgcaatgtatgttttttttttttttacgatttatttactatatgaatgttttgcctgaatacatgcataggtgtcacgtacatgcctgctggaacgcttggaactggagttacaggtggctatgagctacagtgtgagcactgggaatcaaacctgggtcttctgcaagagcaacaaattaaaagtcagctcttaactacttgagctatttttccaactcc

SEQ ID NO: 2 - protein, 309 aa, Mus musculus
MGVPAVPEASSPRWGTLLLAIFLAASRGLVAAFKVTTPYSLYVCPEGQNATLTCRILGPVSKGHDVTIYKTWYLSSRGEVQMCKEHRPIRNFTLQHLQHHGSHLKANASHDQPQKHGLELASDHHGNFSITLRNVTPRDSGLYCCLVIELKNHHPEQRFYGSMELQVQAGKGSGSTCMASNEQDSDSITAAALATGACIVGILCLPLILLLVYKQRQVASHRRAQELVRMDSSNTQGIENPGFETTPPFQGMPEAKTRPPLSYVAQRQPSESGRYLLSDPSTPLSPPGPGDVFFPSLDPVPDSPNSEAI

SEQ ID NO: 3 - DNA, 4714 bp, Homo sapiens
gggggcgggtgcctggagcacggcgctggggccgcccgcagcgctcactcgctcgcactcagtcgcgggaggcttccccgcgccggccgcgtcccgcccgctccccggcaccagaagttcctctgcgcgtccgacggcgacatgggcgtccccacggccctggaggccggcagctggcgctggggatccctgctcttcgctctcttcctggctgcgtccctaggtccggtggcagccttcaaggtcgccacgccgtattccctgtatgtctgtcccgaggggcagaacgtcaccctcacctgcaggctcttgggccctgtggacaaagggcacgatgtgaccttctacaagacgtggtaccgcagctcgaggggcgaggtgcagacctgctcagagcgccggcccatccgcaacctcacgttccaggaccttcacctgcaccatggaggccaccaggctgccaacaccagccacgacctggctcagcgccacgggctggagtcggcctccgaccaccatggcaacttctccatcaccatgcgcaacctgaccctgctggatagcggcctctactgctgcctggtggtggagatcaggcaccaccactcggagcacagggtccatggtgccatgagctgtcaggtgcagacaggcaaagatgcaccatccaactgtgtggtgtacccatcctcctcccaggatagtgaaaacatcacggctgcagccctggctacgggtgcctgcatcgtaggaatcctctgcctccccctcatcctgctcctggtctacaagcaaaggcaggcagcctccaaccgccgtgcccaggagctggtgcggatggacagcaacattcaagggattgaaaaccccggctttgaagcctcaccacctgcccaggggatacccgaggccaaagtcaggcaccccctgtcctatgtggcccagcggcagccttctgagtctgggcggcatctgctttcggagcccagcacccccctgtctcctccaggccccggagacgtcttcttcccatccctggaccctgtccctgactctccaaactttgaggtcatctagcccagctgggggacagtgggctgttgtggctgggtctggggcaggtgcatttgagccagggctggctctgtgagtggcctccttggcctcggccctggttccctccctcctgctctgggctcagatactgtgacatcccagaagcccagcccctcaacccctctggatgctacatggggatgctggacggctcagcccctgttccaaggattttggggtgctgagattctcccctagagacctgaaattcaccagctacagatgccaaatgacttacatcttaagaagtctcagaacgtccagcccttcagcagctctcgttctgagacatgagccttgggatgtggcagcatcagtgggacaagatggacactgggccaccctcccaggcaccagacacagggcacggtggagagacttctcccccgtggccgccttggctcccccgttttgcccgaggctgctcttctgtcagacttcctctttgtaccacagtggctctggggccaggcctgcctgcccactggccatcgccaccttccccagctgcctcctaccagcagtttctctgaagatctgtcaacaggttaagtcaatctggggcttccactgcctgcattccagtccccagagcttggtggtcccgaaacgggaagtacatattggggcatggtggcctccgtgagcaaatggtgtcttgggcaatctgaggccaggacagatgttgccccacccactggagatggtgctgagggaggtgggtggggccttctgggaaggtgagtggagaggggcacctgccccccgccctccccatcccctactcccactgctcagcgcgggccattgcaagggtgccacacaatgtcttgtccaccctgggacacttctgagtatgaagcgggatgctattaaaaactacatggggaaacaggtgcaaaccctggagatggattgtaagagccagtttaaatctgcactctgctgctcctcccccacccccaccttccactccatacaatctgggcctggtggagtcttcgcttcagagccattcggccaggtgcgggtgatgttcccatctcctgcttgtgggcatgccctggctttgtttttatacacataggcaaggtgagtcctctgtggaattgtgattgaaggattttaaagcaggggaggagagtagggggcatctctgtacactctgggggtaaaacagggaaggcagtgcctgagcatggggacaggtgaggtggggctgggcagaccccctgtagcgtttagcaggatgggggccccaggtactgtggagagcatagtccagcctgggcatttgtctcctagcagcctacactggctctgctgagctgggcctgggtgctgaaagccaggatttggggctaggcgggaagatgttcgcccaattgcttggggggttggggggatggaaaaggggagcacctctaggctgcctggcagcagtgagccctgggcctgtggctacagccagggaaccccacctggacacatggccctgcttctaagccccccagttaggcccaaaggaatggtccactgagggcctcctgctctgcctgggctgggccaggggctttgaggagagggtaaacataggcccggagatggggctgacacctcgagtggccagaatatgcccaaaccccggcttctcccttgtccctaggcagaggggggtcccttcttttgttccctctggtcaccacaatgcttgatgccagctgccataggaagagggtgctggctggccatggtggcacacacctgtcctcccagcactttgcagggctgaggtggaaggaccgcttaagcccaggtgttcaaggctgctgtgagctgtgttcgagccactacactccagcctggggacggagcaaaactttgcctcaaaacaaattttaaaaagaaagaaagaaggaaagagggtatgtttttcacaattcatgggggcctgcatggcaggagtggggacaggacacctgctgttcctggagtcgaaggacaagcccacagcccagattccggttctcccaactcaggaagagcatgccctgccctctggggaggctggcctggccccagccctcagctgctgaccttgaggcagagacaacttctaagaatttggctgccagaccccaggcctggctgctgctgtgtggagagggaggcggcccgcagcagaacagccaccgcacttcctcctcagcttcctctggtgcggccctgccctctcttctctggacccttttacaactgaacgcatctgggcttcgtggtttcctgttttcagcgaaatttactctgagctcccagttccatcttcatccatggccacaggccctgcctacaacgcactagggacgtccctccctgctgctgctggggaggggcaggctgctggagccgccctctgagttgccctgggtgcgagaacatggcgcctccagggggcgggaggagcactaggggctggggcaggaggctcctggagcgctggattcctggcacagtctgaggccctgagagggaaatccatgcttttaagaactaattcattgttaggagatcaatcaggaattaggggccatcttacctatctcctgacattcacagtttaatagagacttcctgcctttattccctcccagggagaggctgaaggaatggaattgaaagcaccatttggagggttttgctgacacagcggggactgctcagcactccctaaaaacacaccatggaggccactggtgactgctggtgggcaggctggccctgcctgggggagtccgtggcgatgggcgctggggtggaggtgcaggagccccaggacctgcttttcaaaagacttctgcctgaccagagctcccactacatgcagtggcccagggcagaggggctgatacatggcctttttcagggggtgctcctcgcggggtggacttgggagtgtgcagtgggacagggggctgcaggggtcctgccaccaccgagcaccaacttggcccctggggtcctgcctcatgaatgaggccttccccagggctggcctgactgtgctgggggctgggttaacgttttctcagggaaccacaatgcacgaaagaggaactggggttgctaaccaggatgctgggaacaaaggcctcttgaagcccagccacagcccagctgagcatgaggcccagcccatagacggcacaggccacctggcccattccctgggcattccctgctttgcattgctgcttctcttcaccccatggaggctatgtcaccctaactatcctggaatgtgttgagagggattctgaatgatcaatatagcttggtgagacagtgccgagatagatagccatgtctgccttgggcacgggagagggaagtggcagcatgcatgctgtttcttggccttttctgttagaatacttggtgctttccaacacactttcacatgtgttgtaacttgtttgatccacccccttccctgaaaatcctgggaggttttattgctgccatttaacacagagggcaatagaggttctgaaaggtctgtgtcttgtcaaaacaagtaaacggtggaactacgactaaa

SEQ ID NO: 4 - protein, 311 aa, Homo sapiens
MGVPTALEAGSWRWGSLLFALFLAASLGPVAAFKVATPYSLYVCPEGQNVTLTCRLLGPVDKGHDVTFYKTWYRSSRGEVQTCSERRPIRNLTFQDLHLHHGGHQAANTSHDLAQRHGLESASDHHGNFSITMRNLTLLDSGLYCCLVVEIRHHHSEHRVHGAMELQVQTGKDAPSNCVVYPSSSQDSENITAAALATGACIVGILCLPLILLLVYKQRQAASNRRAQELVRMDSNIQGIENPGFEASPPAQGIPEAKVRHPLSYVAQRQPSESGRHLLSEPSTPLSPPGPGDVFFPSLDPVPDSPNFEVI

SEQ ID NO: 5 - protein, 30 aa, Artificial Sequence
  Consensus sequence for PD-L3
ITAAALATGACIVGILCLPLILLLVYKQRQ

SEQ ID NO: 6 - DNA, 1316 bp, Mus musculus
ggagtcctccccttggagcctgggaggcctagggagaaagtagttctctttcggtggcagggttgctgtcgagggcaccgagcaggaggataggtcgacagagacgaggagttctggctcctcctgcagacatgcaccagcggctgctgggctcgtccctgggrctcgcccccgcgcgggggctctgaatgcctgccgccgcccccatgagagcaccggcctgggctcccgcccctaagcctctgctcgcggagactgagccatgtgggcctggggctgggccgctgcagcgctcctctggctacagactgcaggagccggggcccggcaggagctcaagaagtctcggcagctgtttgcgcgtgtggattcccccaatattaccacgtccaaccgtgagggattcccaggctccgtcaagcccccggaagcctctggacctgagctctcagatgcccacatgacgtggttgaactttgtccgacggccagatgatgggtcctctagaaaacggtgtcgtggccgggacaagaagtcgcgaggcctctcaggtctcccagggcccccaggacctcctggccctcctggtccccctggctcccctggtgtgggcgttaccccagaggccttactgcaggaatttcaggagatactgaaagaggccacagaacttcgattcccagggctaccagacacattgttaccccaggaacccagccaacggctggtggttgaggccttctactgccgtttgaaaggccctgtgctggtggacaagaagactctggtggaactgcaaggattccaagctcctactactcagggcgccttcctgcggggatctggcctgagcctgtccttgggccgattcacagccccagtctctgccatcttccagttttctgccagcctgcacgtggaccacagtgaactgcagggcagaggccggttgcgtacccgggatatggtccgtgttctcatctgtattgagtccttgtgtcatcgtcatacgtccctggaggctgtatcaggtctggagagcaacagcagggtcttcacagtgcaggttcaggggctgctgcatctacagtctggacagtatgtctctgtgttcgtggacaacagttctggggcagtcctcaccatccagaacacttccagcttctcgggaatgcttttgggtacctagcggagctgaagaaacgattgtggattgaggaaccaacaccttgcttcttagaggagctgaaaaggactactcactccccttttaatagttttcatagcaataaagaactccaaacttcttcatcgct

SEQ ID NO: 7 - protein, 308 aa, Mus musculus
MWAWGWAAAALLWLQTAGAGARQELKKSRQLFARVDSPNITTSNREGFPGSVKPPEASGPELSDAHMTWLNFVRRPDDGSSRKRCRGRDKKSRGLSGLPGPPGPPGPPGPPGSPGVGVTPEALLQEFQEILKEATELRFSGLPDTLLPQEPSQRLVVEAFYCRLKGPVLVDKKTLVELQGFQAPTTQGAFLRGSGLSLSLGRFTAPVSAIFQFSASLHVDHSELQGRGRLRTRDMVRVLICIESLCHRHTSLEAVSGLESNSRVFTVQVQGLLHLQSGQYVSVFVDNSSGAVLTIQNTSSFSGMLLGT

SEQ ID NO: 8 - DNA, 1055 bp, Homo sapiens
ctcgccgcgctgagccgcctcgggacggagccatgcggcgctgggcctgggccgcggtcgtggtccccctcgggccgcagctcgtgctcctcgggggcgtcggggcccggcgggaggcacagaggacgcagcagcctggccagcgcgcagatccccccaacgccaccgccagcgcgtcctcccgcgaggggctgcccgaggcccccaagccatcccaggcctcaggacctgagttctccgacgcccacatgacatggctgaactttgtccggcggccggacgacggcgccttaaggaagcggtgcggaagcagggacaagaagccgcgggatctcttcggtcccccaggacctccaggtgcagaagtgaccgcggagactctgcttcacgagtttcaggagctgctgaaagaggccacggagcgccggttctcagggcttctggacccgctgctgccccagggggcgggcctgcggctggtgggcgaggcctttcactgccggctgcagggtccccgccgggtggacaagcggacgctggtggagctgcatggtttccaggctcctgctgcccaaggtgccttcctgcgaggctccggtctgagcctggcctcgggtcggttcacggcccccgtgtccggcatcttccagttctctgccagtctgcacgtggaccacagtgagctgcagggcaaggcccggctgcgggcccgggacgtggtgtgtgttctcatctgtattgagtccctgtgccagcgccacacgtgcctggaggccgtctcaggcctggagagcaacagcagggtcttcacgctacaggtgcaggggctgctgcagctgcaggctggacagtacgcttctgtgtttgtggacaatggctccggggccgtcctcaccatccaggcgggctccagcttctccgggctgctcctgggcacgtgagggcgcccaggggggctggcgaggagctgccgccggatcccggggaccctcctactgatgcccgtggtcaccacaataaagagccctccaccctcaaaaaaaaaaaaaaaaaaa

SEQ ID NO: 9 - protein, 302 aa, Homo sapiens
MRRWAWAAVVVLLGPQLVLLGGVGARREAQRTQQPGQRADPPNATASASSREGLPEAPKPSQASGPEFSDAHMTWLNFVRRPDDGALRKRCGSRDKKPRDLFGPPGPPGAEVTAETLLHEFQELLKEATERRFSGLLDPLLPQGAGLRLVGEAFHCRLQGPRRVDKRTLVELHGFQAPAAQGAFLRGSGLSLASGRFTAPVSGIFQFSASLHVDHSELQGKARLRARDVVCVLICIESLCQRHTCLEAVSGLESNSRVFTLQVQGLLQLQAGQYASVFVDNGSGAVLTIQAGSSFSGLLLGT

SEQ ID NO: 10 - protein, 17 aa, Artificial Sequence
  Consensus sequence for Treg-sTNF
IFQFSASLHVDHSELQG

SEQ ID NO: 11 - protein, 112 aa, Homo sapien
  MISC_FEATURE (1)..(112): PD1L1 Ig-V domain
FTITAPKDLYVVEYGSNVTMECRFPVERELDLLALVVYWEKEDEQVIQFVAGEEDLKPQHSNFRGRASLPKDQLLKGNAALQITDVKLQDAGVYCCIISYGGADYKRITLKV

SEQ ID NO: 12 - protein, 99 aa, Homo sapien
  MISC_FEATURE (1)..(99): PD1L2 Ig-V domain
FTVTAPKEVYTVDVGSSVSLECDFDRRECTELEGIRASLQKVENDTSLQSERATLLEEQLPLGKALFHIPSVQVRDSGQYRCLVICGAAWDYKYLTVKV

SEQ ID NO: 13 - protein, 113 aa, Homo sapien
  MISC_FEATURE (1)..(113): B7H4 Ig-V domain
HFITVTTFTSAGNIGEDGTLSCTFEPDIKLNGIVIQWLKEGIKGLVHEFKEGKDDLSQQHEMFRGRTAVFADQVVVGNASLRLKNVQLTDAGTYTCYIRTSKGKGNANLEYKT

SEQ ID NO: 14 - protein, 110 aa, Homo sapien
  MISC_FEATURE (1)..(110): B7H3 Ig-V domain
VEVQVSEDPVVALVDTDATLRCSFSPEPGFSLAQLNLIWQLTDTKQLVHSFTEGRDQGSAYSNRTALFPDLLVQGNASLRLQRVRVTDEGSYTCFVSIQDFDSAAVSLQV

SEQ ID NO: 15 - protein, 136 aa, Homo sapien
  MISC_FEATURE (1)..(136): VISTA Ig-V domain
FKVTTPYSLYVCPEGQNATLTCRILGPVSKGHDVTIYKTWYLSSRGEVQMCKEHRPIRNFTLQHLQHHGSHLKANASHDQPQKHGLELASDHHGNFSLTLRNVTPRDSGLYCCLVIELKNHHPEQRFYGSMELQVQ

SEQ ID NO: 16 - protein, 311 aa, Homo sapiens; identical to SEQ ID NO: 4

SEQ ID NO: 17 - protein, 309 aa, Mus musculus; identical to SEQ ID NO: 2
  misc-feature (1)..(309): VISTA orthologue

SEQ ID NO: 18 - protein, 312 aa, Kangaroo
  misc_feature (1)..(312): VISTA orthlogue
MNVPTSVLESGGRRWGPLLLAFFLAASRGLVAAFKVATPYSLYVCPEGENITLACQLLGPVPKGHDVSFYKTWFRSSRGEVQVCSEHRPIRNVTLQNLHPYHGGHQASNTSHNLLQSHGLETASDHHGNFSITMRNLTVQDGGLYCCLVVEMRHRHSEHRVHAAMELQVQKGKDAPSKCITYPSSPEESDNITAAALATGACIVGILCLPLILLLVYKQRQVASHRRAQELVRMDSSPQGIENPGFEAPPSSQGLPEAKVRPPLSYMAQRQPSESGRHLLSEPNTPLSPPGPGDVFFPSLDPVPDSPNSEFN

SEQ ID NO: 19 - protein, 310 aa, Dolphin
  misc_feature (1)..(310): VISTA orthologue
MGVPPVPEAGSWRRGPVLLAFFLAASRGLVAAFKVATPYSLYVCPEGQNVTLTCRLLGPLAKGHDVTFYKTWYRSSRGEVQACSERRPIRNLTFQDLHLHHGGHQANSSQDLAQRHGLESASDHHGNFTITMRNLTLLDGGLYCCLVVEIRHRHSEQRLYGAMELQVQRGEEAPSKCTVYPPSSKESESITAAALATSACIVGILCLPLILLLVYKQRQVASNRRAQELVRMDSNTQGIENPGFETSPPSHGMPETKPRQPLTYMARRQPSESGRHLLSEPNTPLSPPGPGDVFFPSLDPVPDSPNSEAI

SEQ ID NO: 20 - protein, 288 aa, Gallus gallus
  misc_feature (1)..(288): VISTA orthlogue
GGTAAFLVTVPYTLCICPEGQNVTLSCRVSGPPADHHDLIFKTWYFSNNGDQSCSEKRHVRNLTEKELRHDPGRHHSTAANSTARSPHGSLASHHGVEFVPDHHGAFHIVVMNLTLQDSGNYCCYAMETRRDHGKAHTLHIAHGFVELQIQRGRGSLQNCTFHTATSKDITAAALATGACIVGILCLPLILLLIYKQRQAVSHRRAHELVRMESSAQGIENPVFEALPAGSTEQRPRPQLSYLGGRQLSESGRHLLSEPNTPLSPPAPGECFFPTLDPVPDSPNSLKA

SEQ ID NO: 21 - protein, 260 aa, Xenopus
  misc_feature (1)..(260): VISTA orthologue
DAITAFSVSALYSHITCPEGQNVNLTCTVSGHVADKHDVLFSLWHFSKDKNSNCLERRHIQNTTERDHLHKEHLSHSMHNGAFQITLTNVSQQDSGGYCCYVIEASKKHHTRHYSYIEFQVKTDDLNLYTCMFHSPTEGDNSSTAAALAIVSCVIGILCMPLLLFLVYKQRRALSHRRSYHFVFIDFSEAQGIENPVFDDPPPANVVEQRPRLAFMASRQQSESDRHLLSEPNTPLSPSCPNECFFPSLPVPDSPDPGNV

SEQ ID NO: 22 - protein, 315 aa, Taeniopygia guttata
  misc_feature (1)..(315): VISTA orthologue
GHPATMGTASPRPGLLLAALCLLASHGGADAFLISTPYSLCVCPEGQNVTLSCRISGALAERHDLLYKTWYFSSTGDQSCSDKRHIRNVTDKELRHDLGRHHELPGNASQKPPFGWQSGHHGVELVLDHHGAFHLVVMNLTLQDSGNYCCYAVEVRREGHSKPHTVQAAHGFVELQIQRGEPCSHARAQSQRAADDITAAVLATGACIVGILCLPLILLLIYKQRQAASSRRAHELVRMDSGAQGIENPVFEAVPSAGAEPRPRAQLSYVASRLPSESGRHLLSEPSTPLSPPGPGDCFFPTLDPVPDSPNSLKA

SEQ ID NO: 23 - protein, 274 aa, Danio rerio
  misc_feature (1)..(274): VISTA orthologue
MDVFRAVLLCFHVFTAIQASGDHHSLRVSVPHRTYECPEGADVILKCVPSGTKAYPQDTFWTTWLYTPRSQDHCQKGAHPRKANHTNRSLGVVYSSGDKVFSVSLKNVKHTDQGKYCCWLLDLHGRHKEQEAHDFMYLSVMPTPKDAHNGSLKCLEYSHTASDDVAEGLAIAACVAFVLCLPLILMLVYRQRQTVERHRRAHELVRMDSEAQGHENPVFLGDSPEPKMRTVSQIMMRQPSETGHHLLSEPGTPFSPNIQGELFFSAQGLPESNI

SEQ ID NO: 24 - protein, 293 aa, Fugu
  misc_feature (1)..(293): VISTA orthologue
LEKFTSAHHTKQTLEKGLNLLCLTKSNAHHGHPAMSVSASHLYYTCPEGANATLVCNQRGGALHPNDSLWRLWFFTPHKDQHCTKHGPRNVTFKHSKLSSGLHFGATQENFWVQLQNVTHADQGRYCCAALEIESIHHEAVQRTHSHMFLNIIPRGTGSPNCTVSAPSAPEGNATLCTVPVALAMGACILALLSLPLILLLVYRQRQSAQSRRRAQELVRMDSEAHGHENPVFLGGSPQIKNRTVSQIMARQSSETGRHLLSEPGTPLSPPAHGDVFFPAEDTIFETPELRQV

SEQ ID NO: 25 - protein, 159 aa, Homo sapien
  DOMAIN (1)..(159): Extracellular domain
FKVTTPYSLYVCPEGQNATLTCRILGPVSKGHDVTIYKTWYLSSRGEVQMCKEHRPIRNFTLQHLQHHGSHLKANASHDQPQKHGLELASDHHGNFSITLRNVTPRDSGLYCCLVIELKNHHPEQRFYGSMELQVQAGKGSGSTCMASNEQDSDSITAA

SEQ ID NO: 26 - protein, 221 aa, Homo sapien
  DOMAIN (1)..(221): Extracellular domain
FTITAPKDLYVVEYGSNVTMECRFPVERELDLLALVVYWEKEDEQVIQFVAGEEDLKPQHSNFRGRASLPKDQLLKGNAALQITDVKLQDAGVYCCIISYGGADYKRITLKVNAPYRKINQRISVDPATSEHELICQAEGYPEAEVIWTNSDHQPVSGKRSVTTSRTEGMLLNVTSSLRVNATANDVFYCTFWRSQPGQNHTAELIIPELPATHPPQNRTH

SEQ ID NO: 27 - protein, 202 aa, Homo sapien
  DOMAIN (1)..(202): Extracellular domain
LFTVTAPKEVYTVDVGSSVSLECDFDRRECTELEGIRASLQKVENDTSLQSERATLLEEQLPLGKALFHIPSVQVRDSGQYRCLVICGAAWDYKYLTVKVKASYMRIDTRILEVPGTGEVQLTCQARGYPLAEVSWQNVSVPANTSHIRTPEGLYQVTSVLRLKPQPSRNFSCMFWNAHMKELTSAIIDPLSRMEPKVPRTW

SEQ ID NO: 28 - protein, 220 aa, Homo sapien
  DOMAIN (1)..(220): Extracellular domain
VEVQVSEDPVVALVDTDATLFCSFSPEPGFSLAQLNLIWQLTDTKQLVHSFTEGRDQGSAYSNRTALFPDLLVQGNASLRLQRVRVTDEGSYTCTVSIQDFDSAAVSLQVAAPYSKPSMTLEPNKDLRPGNMVTITCSSYQGYPEAEVFWKDGQGVPLTGNVTTSQMANERGLFDVHSVLRVVLGANGTYSCLVRNPVLQQDAHGSVTITGQPLTFPPEA

SEQ ID NO: 29 - protein, 233 aa, Homo sapien
  DOMAIN (1)..(233): Extracellular domain
LIIGFGISGKHFITVTTFTSAGNIGEDGTLSCTFEPDIKLNGIVIQWLKEGIKGLVHEFKEGKDDLSQQMEMFAGRTAVFADQVVVGNASLRLKNVQLTDAGTYTCYIRTSKGKGNANLEYKTGAFSMPEINVDYNASSESLRCEAPRWFPQPTVAWASQVDQGANFSEVSNTSFELNSENVTMKVVSVLYNVTINNTYSCMIENDIAKATGDIKVTDSEVKRRSQLQLLNSG

SEQ ID NO: 30 - protein, 159 aa, Mus musculus
  DOMAIN (1)..(159): Extracellular domain
FKVTTPYSLYVCPEGQNATLTCRILGPVSKGHDVTIYKTWYLSSRGEVQMCKEHRPIRNFTLQHLQHHGSHLKANASHDQPQKHGLELASDHHGNFSITLRNVTPRDSGLYCCLVIELKNHHPEQRFYGSMELQVQAGKCSGSTCMASNEQDSDSITAA

SEQ ID NO: 31 - protein, 149 aa, Homo sapien
  Domain (1)..(149): Extracellular domain
SGWLLEVPNGPWRSLTFYPAWLTVSEGANATFTCSLSNWSEDLMLNWNRLSPSNQTEKQAAFCNGLSQPVQDARFQIIQLPNRHDFHMNILDTRRNDSGIYLCGAISLMPKAKIEESPGAELVVTERILETSTRYPSPSPKPEERFQGM

SEQ ID NO: 32 - protein, 126 aa, Homo sapien
  Domain (1)..(126): Extracellular domain
EAIQVTQPSVVLASSHGVASFPCEYSPSHNTDEVRVTVLRQTNDQMTEVCATTFTEKNTVGFLDYPFCSGTFNESRVNLTIQGLRAVDTGLYLCKVELMYPPPYFVGMGNGTQIYVIDPEPCPDSD

SEQ ID NO: 33 - protein, 71 aa, Homo sapien
  Domain (1)..(71): Extracellular domain
RSNAEFNCDGDFDNETVTFRLWNLHVNHTDIYFCKIEFMYPPPYLDNERSNGTITHIKEKHLCHTQSSPKL

SEQ ID NO: 34 - protein, 154 aa, Homo sapien
  domain (1)..(154): Extracellular domain
EKATKRNDEECPVQLTITRNSKQSARTGELFKIQCPVKYCVHRPNVTWCKHNGTICVPLEVSPQLYTSWEENQSVPVFVLHFKPIHLSDNGSYSCSTNFNSQVINSHSVTIHVRERTQNSSEHPLITVSDIPDATNASGPSTMEERPGRTWLLY

SEQ ID NO: 35 - protein, 124 aa, Homo sapien
  Domain (1)..(124): Extracellar domain
EINGSADHRMFSFHNGGVQISCKYPETVQQLKMRLFREREVLCELTKTKGSGNAVSIKNPMLCLYMLSNNSVSFFLNNPDSSQGSYYFCSLSIFDPPPFQERNLSGGYLHIYESQLCCQLKLWL

SEQ ID NO: 36 - protein, 306 aa, Mus musculus
MGVPNVPEASSPRWGTLILADFLAASRGLVAAFKVTTPYSLYVCPEGQNATLTCRILGPVSKGHDVTIYKTWYLSSRGEVQMCKEERPIRNFILQHLQHHGSHLKANASHDQPQKHGLETASDHHGNFSITLRNVTPRDSGLYCCLVIELKNHHPKQRFYGSMELQVQAGKGSGTNASNEQDSDSITAAALATGACIVGILCLPLILLLVYKQRQVASHRRAQELVRMDSSNTQGIKNPGFETTPPFQGMPEAKTRPPLSYVAQRQPSESGRYLLSDPSTPLSPPGPGDVFFPSLDPVPDSNSEAI

SEQ ID NO: 37 - protein, 308 aa, Homo sapien
MGVPTAIEASSWRWGSLIFALFLAASLGPVAAFKVATPYSLVVCPEGQNVTLTCRLLGPVDKGHDVTFYKTWYRSSRGEVQTCSERRPIRNLTFQDLKLHHGGHQAANTSHDLAQRHGLESASDHHGNFSITNRNLTLLDSGLYCCLVVEIRHHHSKHRVHGAMELQVQTGKDAPNVVYPSSSQDSENITAAALATGACIVGILCLPLILLLVYKQRQAASNRRAQELVRMDSNIQGIKNPGFEASPPAQGIPEAKVRHPLSYVAQRQPSESGRHLLSEPSTPLSPPGPGDVFFPSLDPVPDSNFEVI

SEQ ID NO: 38 - DNA, 25 bp, Artificial Sequence
  siRNA
gggcacgatgtgaccttctacaaga

SEQ ID NO: 39 - DNA, 25 bp, Artificial Sequence
  siRNA
cagatgccaaatgacttacatctta

SEQ ID NO: 40 - DNA, 25 bp, Artificial Sequence
  siRNA
gagatggattgtaagagccagttta

SEQ ID NO: 41 - DNA, 25 bp, Artificial Sequence
  siRNA
gggctttgaggagagggtaaacata

SEQ ID NO: 42 - DNA, 25 bp, Artificial Sequence
  siRNA
cctatctcctgacattcacagttta

SEQ ID NO: 43 - DNA, 25 bp, Artificial Sequence
  siRNA
cagtttaatagagacttcctgcctt

SEQ ID NO: 44 - DNA, 25 bp, Artificial Sequence
  siRNA
cagggagaggctgaaggaatggaat

SEQ ID NO: 45 - DNA, 25 bp, Artificial Sequence
  siRNA
ggaatgtgttgagagggattctgaa

SEQ ID NO: 46 - DNA, 25 bp, Artificial Sequence
  siRNA
gagagggattctgaatgatcaatat

SEQ ID NO: 47 - DNA, 25 bp, Artificial Sequence
  siRNA
cacagagggcaatagaggttctgaa

SEQ ID NO: 48 - DNA, 25 bp, Artificial Sequence
  siRNA
cagatgccaaatgacttacatctta

SEQ ID NO: 49 - DNA, 25 bp, Artificial Sequence
  siRNA
gagatggattgtaagagccagttta

SEQ ID NO: 50 - DNA, 25 bp, Artificial Sequence
  siRNA
ggtgagtcctctgtggaattgtgat

SEQ ID NO: 51 - DNA, 25 bp, Artificial Sequence
  siRNA
gggctttgaggagagggtaaacata

SEQ ID NO: 52 - DNA, 25 bp, Artificial Sequence
  siRNA
cctatctcctgacattcacagttta

SEQ ID NO: 53 - DNA, 25 bp, Artificial Sequence
  siRNA
cagtttaatagagacttcctgcctt

SEQ ID NO: 54 - DNA, 25 bp, Artificial Sequence
  siRNA
cagggagaggctgaaggaatggaat

SEQ ID NO: 55 - DNA, 25 bp, Artificial Sequence
  siRNA
ggaatgtgttgagagggattctgaa

SEQ ID NO: 56 - DNA, 25 bp, Artificial Sequence
  siRNA
gagagggattctgaatgatcaatat

SEQ ID NO: 57 - DNA, 25 bp, Artificial Sequence
  siRNA
cacagagggcaatagaggttctgaa

SEQ ID NO: 58 - DNA, 25 bp, Artificial Sequence
  siRNA
acaaagggcacgatgtgaccttcta

SEQ ID NO: 59 - DNA, 25 bp, Artificial Sequence
  siRNA
gggcacgatgtgaccttctacaaga

SEQ ID NO: 60 - DNA, 25 bp, Artificial Sequence
  siRNA
gaccaccatggcaacttctccatca

SEQ ID NO: 61 - DNA, 25 bp, Artificial Sequence
  siRNA
cagacaggcaaagatgcaccatcca

SEQ ID NO: 62 - DNA, 25 bp, Artificial Sequence
  siRNA
ggcaaagatgcaccatccaactgtg

SEQ ID NO: 63 - DNA, 25 bp, Artificial Sequence
  siRNA
ccatccaactgtgtggtgtacccat

SEQ ID NO: 64 - DNA, 25 bp, Artificial Sequence
  siRNA
ggatggacagcaacattcaagggat

SEQ ID NO: 65 - DNA, 25 bp, Artificial Sequence
  siRNA
gacagcaacattcaagggattgaaa

SEQ ID NO: 66 - DNA, 25 bp, Artificial Sequence
  siRNA
ccctgtccctgactctccaaacttt

SEQ ID NO: 67 - DNA, 25 bp, Artificial Sequence
  siRNA
cctgactctccaaactttgaggtca

SEQ ID NO: 68 - protein, 457 aa, Artificial Sequence
  Human VISTA - human IgG1 Fc fusion protein CDM8
  X (61)..(61): unsure
  X (63)..(63): unsure
  X (200)..(200): unsure
  X (202)..(202): unsure
  X (239)..(239): unsure
  X (259)..(259): unsure
  X (270)..(270): unsure
  X (278)..(278): unsure
  X (279)..(279): unsure
  X (281)..(281): unsure
  X (282)..(282): unsure
  X (284)..(284): unsure
  X (287)..(287): unsure
  X (288)..(288): unsure
  X (291)..(291): unsure
  X (292)..(292): unsure
  X (299)..(299): unsure
  X (312)..(312): unsure
  X (319)..(319): unsure
  X (330)..(330): unsure
  X (339)..(339): unsure
  X (350)..(350): unsure
  X (351)..(351): unsure
  X (354)..(354): unsure
  X (356)..(356): unsure
  X (360)..(360): unsure
  X (373)..(373): unsure
  X (376)..(376): unsure
MSLLFALFLAASLGPVAAFKVATPYSLYVCPEGQNVTLTCRLLGPVDKGHDVTFYKTWYRXSXGEVQTCSERRPIRNLTFQDLHLHHGGHQAANTSHDLAQRHGLESASDHHGNFSITMRNLTLLDSGLYCCLVVEIRHHHSEHRVHGAMELQVQTGKDAPSNCVVYPSSSQESENITAADPGGGGGRLVPRGFGTGDPXPXSSDKTHTCPPCPAPDSRVHRQSSSSPKTKDTLMISRXPEVTCVVVDVSQEDPEVKFXWYVDGVEMHRXKTKPREEXXNXXLXMGXXLTXXQQDWLNXKDYKFKVSNKKQXNPFEKTXSKSKRQTREPXVYNLPPSRXELTKIQVSLTXXVKXFXPSDXAVEWESNGQPENXYKXTPPVLDSDGSFFLYSKLTVDKSRWQQGNVFSCSVMHEALHNHYTQKSLSLSPGKGSAGGSGGLNDIFEAQKIEWHESRGSL

SEQ ID NO: 69 - protein, 415 aa, Artificial Sequence
  Human VISTA - Human IgG1 Fc fusion protein pFUSE-hIgG1e3-Fc2
MYRMQLLSCIALSLALVTNSFKVATPYSLYVCPEGQNVTLTCRLLGPVDKGHDVTFYKTWYRSSRGEVQTCSERRPIRNLTFQDLHLHHGGHQAANTSHDLAQRHGLESASDHHGNFSITMRNLTLLDSGLYCCLVVEIRHHHSEHRVHGAMELQVQTGKDAPSNCVVYPSSSQDSENITAAARSISAMVRSVECPPCPAPPVAGPSVFLFPPKPKDTLMISRTPEVTCVVVDVSHEDPEVKFNWYVDGVEVHNAKTKPREEQYNSTYRVVSVLTVLHQDWLNGKEYKCKVSNKGLPSSIEKTISKAKGQPREPQVYTLPPSREEMTKNQVSLTCLVKGFYPSDIAVEWESNGQPENNYKTTPPVLDSDGSFFLYSKLTVDKSRWQQGNVFSCSVMHEALHNHYTQKSLSLSPGK

SEQ ID NO: 70 - protein, 203 aa, Artificial Sequence
  VISTA Ig fusion protein Fc domain concensus
  X (3)..(3): T or P
  X (12)..(12): unsure
  X (24)..(24): unsure
  X (32)..(32): unsure
  X (40)..(40): unsure
  X (42)..(42): unsure
  X (43)..(43): unsure
  X (51)..(52): unsure
  X (54)..(55): unsure
  X (56)..(56): L or Y
  X (57)..(57): unsure
  X (58)..(58): M or V
  X (59)..(59): G or V
  X (60)..(61): unsure
  X (64)..(65): unsure
  X (66)..(66): Q or H
  X (72)..(72): unsure
  X (74)..(74): D or E
  X (77)..(77): F or C
  X (83)..(83): K or G
  X (84)..(84): Q or L
  X (85)..(85): unsure
  X (86)..(86): N or S
  X (87)..(87): P or S
  X (88)..(88): F or I
  X (92)..(92): unsure
  X (95)..(95): S or A
  X (97)..(97): R or G
  X (99)..(99): T or P
  X (103)..(103): unsure
  X (106)..(106): N or T
  X (112)..(112): unsure
  X (114)..(114): L or M
  X (117)..(117): I or N
  X (123)..(124): unsure
  X (127)..(127): unsure
  X (129)..(129): unsure
  X (133)..(133): unsure
  X (146)..(146): unsure
  X (149)..(149): unsure
PKXKDTLMISRXPEVTCVVVDVSXEDPEVKFXWYVDGVEXHXXKTKPREEXXNXXXXXXXXLTXXXQDWLNXKXYKXKVSNKXXXXXXEKTXSKXKXQXREPXVYXLPPSRXEXTKXQVSLTXXVKXFXPSDXAVEWESNGQPENXYKXTPPVLDSDGSFFLYSKLTVDKSRWQQGNVFSCSVMHEALHNHYTQKSLSLSPGK

SEQ ID NO: 71 - protein, 19 aa, Artificial Sequence
  Serine-glycine linker
GTSGSSGSGSGGSGSGGGG

SEQ ID NO: 72 - protein, 427 aa, Artificial Sequence
  VISTA Ig fusion protein with serine-glycine linker
MYRMQLLSCIALSLALVTNSFKVATPYSLYVCPEGQNVTLTCRLLGPVDKGHDVTFYKTWYRSSRGEVQTCSERRPIRNLTFQDLHLHHGGHQAANTSHDLAQRHGLESASDHHGNFSITMRNLTLLDSGLYCCLVVEIRHHHSEHRVHGAMELQVQTGKDAPSNCVVYPSSSQDSENITAAAGTSGSSGSGSGGSGSGGGGRSVECPPCPAPPVAGPSVFLFPPKPKDTLMISRTPEVTCVVVDVSHEDPEVKFNWYVDGVEVHNAKTKPREEQYNSTYRVVSVLTVLHQDWLNGKEYKCKVSNKGLPSSIEKTISKAKGQPREPQVYTLPPSREEMTKNQVSLTCLVKGFYPSDIAVEWESNGQPENNYKTTPPVLDSDGSFFLYSKLTVDKSRWQQGNVFSCSVMHEALHNHYTQKSLSLSPGK

SEQ ID NO: 73 - protein, 484 aa, Artificial Sequence
  VISTA-Ig fusion protein
MPMGSLQPLATLYLLGMLVASCLGTSMSLLFALFLAASLGPVAAFKVATPYSLYVCPEGQNVTLTCRLLGPVDKGHDVTFYKTWYRSSRGEVQTCSERRPIRNLTFQDLHLHHGGHQAANTSHDLAQRHGLESASDHHGNFSITMRNLTLLDSGLYCCLVVDIRHHHSEHRVHGAMELQVQTGKDAPSNCVVYPSSSQESENITAADPGGGGGRLVPRGFGTGDPEPKSSDKTHTCPPCPAPEFEGAPSVFLFPPKPKDTLMISRTPEVTCVVVDVSHEDPEVKFNWYVDGVEVHNAKTKPREEQYNSTYRVVSVLTVLHQDWLNGKEYKCKVSNKALPTPIEKTISKAKGQPREPQVYTLPPSRDELTKNQVSLTCLVKGFYPSDIAVEWESNGQPENNYKTTPPVLDSDGSFFLYSKLTVDKSRWQQGNVFSCSVMHEALHNHYTQKSLSLSPGKGSAGGSGGLNDIFEAQKIEWHESRGSL

SEQ ID NO: 74 - protein, 232 aa, Artificial Sequence
  Human IgG1 concensus sequence
  X (5)..(5): S or C
  X (19)..(19): F or L
  X (20)..(20): E or L
  X (22)..(22): A or G
  X (115)..(115): T or A
  X (141)..(141): D or E
  X (143)..(143): L or M
EPKSXDKTHTCPPCPAPEXXGXPSVFLFPPKPKDTLMISRTPEVTCVVVDVSHEDPEVKFNWYVDGVEVHNAKTKPREEQYNSTYRVVSVLTVLHQDWLNGKEYKCKVSNKALPXPIEKTISKAKGQPREPQVYTLPPSRXEXTKNQVSLTCLVKGFYPSDIAVEWESNGQPENNYKTTPPVLDSDGSFFLYSKLTVDKSRWQQGNVFSCSVMHEALHNHYTQKSLSLSPGK

SEQ ID NO: 75 - protein, 413 aa, Artificial Sequence
  Human VISTA Ig construct
FKVATPYSLYVCPEGQNVTLTCRLLGPVDKGHDVTFYKTWYRSSRGEVQTCSERRPIRNLTFQDLHLHHGGHQAANTSHDLAQRHGLESASDHHGNFSITMRNLTLLDSGLYCCLVVDIRHHHSEHRVHGAMELQVQTGKDAPSNCVVYPSSSQESENITAADPGGGGGRLVPRGFGTGDPEPKSSDKTHTCPPCPAPEFEGAPSVFLFPPKPKDTLMISRTPEVTCVVVDVSHEDPEVKFNWYVDGVEVHNAKTKPREEQYNSTYRVVSVLTVLHQDWLNGKEYKCKVSNKALPTPIEKTISKAKGQPREPQVYTLPPSRDELTKNQVSLTCLVKGFYPSDIAVEWESNGQPENNYKTTPPVLDSDGSFFLYSKLTVDKSRWQQGNVFSCSVMHEALHNHYTQKSLSLSPGK